European Patent Specification EP 3 565 568 B1, published August 6, 2025. Title: ALTERED VIRUS. Applicant: Replimune Limited. The sequence listing filed with the application follows.

SEQUENCE LISTING (46 sequences)

SEQ ID NO: 1 - protein, 108 aa, Homo sapiens
IVLTQSPGTLSLSPGERATLSCRASQSVGSSYLAWYQQKPGQAPRLLIYGAFSRATGIPDRFSGSGSGTDFTLTISRLEPEDFAVYYCQQYGSSPWTFGQGTKVEIKR

SEQ ID NO: 2 - protein, 215 aa, Homo sapiens
EIVLTQSPGTLSLSPGERATLSCRASQSVGSSYLAWYQQKPGQAPRLLIYGAFSRATGIPDRFSGSGSGTDFTLTISRLEPEDFAVYYCQQYGSSPWTFGQGTKVEIKRTVAAPSVFIFPPSDEQLKSGTASVVCLLNNFYPREAKVQWKVDNALQSGNSQESVTEQDSKDSTYSLSSTLTLSKADYEKHKVYACEVTHQGLSSPVTKSFNRGEC

SEQ ID NO: 3 - protein, 118 aa, Homo sapiens
QVQLVESGGGVVQPGRSLRLSCAASGFTFSSYTMHWVRQAPGKGLEWVTFISYDGNNKYYADSVKGRFTISRDNSKNTLYLQMNSLRAEDTAIYYCARTGWLGPFDYWGQGTLVTVSS

SEQ ID NO: 4 - protein, 103 aa, Homo sapiens
ASTKGPSVFPLAPSSKSTSGGTAALGCLVKDYFPEPVTVSWNSGALTSGVHTFPAVLQSSGLYSLSSVVTVPSSSLGTQTYICNVNHKPSNTKVDKRVEPKSC

SEQ ID NO: 5 - protein, 227 aa, Homo sapiens
DKTHTCPPCPAPELLGGPSVFLFPPKPKDTLMISRTPEVTCVVVDVSHEDPEVKFNWYVDGVEVHNAKTKPREEQYNSTYRVVSVLTVLHQDWLNGKEYKCKVSNKALPAPIEKTISKAKGQPREPQVYTLPPSRDELTKNQVSLTCLVKGFYPSDIAVEWESNGQPENNYKTTPPVLDSDGSFFLYSKLTVDKSRWQQGNVFSCSVMHEALHNHYTQKSLSLSPGK

SEQ ID NO: 6 - protein, 448 aa, Homo sapiens
QVQLVESGGGVVQPGRSLRLSCAASGFTFSSYTMHWVRQAPGKGLEWVTFISYDGNNKYYADSVKGRFTISRDNSKNTLYLQMNSLRAEDTAIYYCARTGWLGPFDYWGQGTLVTVSSASTKGPSVFPLAPSSKSTSGGTAALGCLVKDYFPEPVTVSWNSGALTSGVHTFPAVLQSSGLYSLSSVVTVPSSSLGTQTYICNVNHKPSNTKVDKRVEPKSCDKTHTCPPCPAPELLGGPSVFLFPPKPKDTLMISRTPEVTCVVVDVSHEDPEVKFNWYVDGVEVHNAKTKPREEQYNSTYRVVSVLTVLHQDWLNGKEYKCKVSNKALPAPIEKTISKAKGQPREPQVYTLPPSRDELTKNQVSLTCLVKGFYPSDIAVEWESNGQPENNYKTTPPVLDSDGSFFLYSKLTVDKSRWQQGNVFSCSVMHEALHNHYTQKSLSLSPGK

SEQ ID NO: 7 - protein, 21 aa, Mus musculus
METDTLLLWVLLLWVPGSTGD

SEQ ID NO: 8 - protein, 15 aa, Artificial Sequence
  (Gly4Ser)3 linker
GGGGSGGGGSGGGGS

SEQ ID NO: 9 - protein, 489 aa, Homo sapiens
METDTLLLWVLLLWVPGSTGDIVLTQSPGTLSLSPGERATLSCRASQSVGSSYLAWYQQKPGQAPRLLIYGAFSRATGIPDRFSGSGSGTDFTLTISRLEPEDFAVYYCQQYGSSPWTFGQGTKVEIKRGGGGSGGGGSGGGGSQVQLVESGGGVVQPGRSLRLSCAASGFTFSSYTMHWVRQAPGKGLEWVTFISYDGNNKYYADSVKGRFTISRDNSKNTLYLQMNSLRAEDTAIYYCARTGWLGPFDYWGQGTLVTVSSDKTHTCPPCPAPELLGGPSVFLFPPKPKDTLMISRTPEVTCVVVDVSHEDPEVKFNWYVDGVEVHNAKTKPREEQYNSTYRVVSVLTVLHQDWLNGKEYKCKVSNKALPAPIEKTISKAKGQPREPQVYTLPPSREEMTKNQVSLTCLVKGFYPSDIAVEWESNGQPENNYKTTPPVLDSDGSFFLYSKLTVDKSRWQQGNVFSCSVMHEALHNHYTQKSLSLSPGK

SEQ ID NO: 10 - DNA, 1470 bp, Homo sapiens
atggaaactgacaccctgctgctgtgggtcctgctgctgtgggtgcctggatccaccggcgatatcgtgctgacccagtctcctggcacactgagtctgtcaccaggggagcgagcaacactgtcttgtagagccagccagtctgtgggaagctcctacctggcttggtatcagcagaagccaggccaggcacccaggctgctgatctacggagccttcagccgggccactggcattccagacaggttctctggaagtggctcagggaccgacttcaccctgaccatcagccgactggagcccgaagacttcgccgtgtactattgccagcagtacggctctagtccttggacttttggacagggcaccaaagtggagatcaagcgcggcgggggaggctctgggggaggcgggagtggaggcgggggatcacaggtccagctggtggaaagcggcgggggagtggtccagccaggccggagcctgcggctgagctgcgccgcttcaggattcacattttcaagctataccatgcactgggtccggcaggcaccagggaagggactggagtgggtgaccttcatcagctatgacggcaacaacaagtattacgctgattccgtgaaagggaggtttaccattagccgcgacaactccaaaaatacactgtacctgcagatgaacagcctgcgggccgaggatactgctatctactattgcgcaagaaccgggtggctgggacccttcgactattggggccaggggactctggtcaccgtgtcctctgataagacacacacatgccctccctgtcctgcaccagagctgctgggcgggccatccgtgttcctgtttccacccaagcctaaagacaccctgatgatcagccggacacctgaagtcacttgcgtggtcgtggacgtgagtcacgaggatccagaagtcaagtttaactggtacgtggatggcgtcgaggtgcataatgccaagaccaaacctcgcgaggaacagtacaatagcacatatcgagtcgtgtccgtcctgactgtgctgcatcaggattggctgaacggcaaagagtataagtgcaaagtgagcaataaggcactgcctgccccaatcgagaaaacaatttccaaggctaaaggccagcccagggaacctcaggtgtacactctgcctccaagtcgcgaggaaatgaccaagaaccaggtgagcctgacctgtctggtgaaagggttctatccatcagacattgcagtggagtgggaaagcaatggacagcccgaaaacaattacaagaccacaccccctgtgctggacagcgatggctccttctttctgtattctaagctgactgtggataaaagtcgctggcagcaggggaacgtctttagctgttccgtgatgcatgaggctctgcacaatcattacacacagaagtctctgagtctgtcacccggcaaatga

SEQ ID NO: 11 - protein, 127 aa, Mus musculus
IRRADIVMTQTTLSLPVSLGDQASISCRSSQSIVHSNGNTYLEWYLQKPGQSPKLLIYKVSNRFSGVPDRFSGSGSGTDFTLKISRVEAEDLGVYYCFQGSHVPYTFGGGTKLEIKRADAAPTVSGS

SEQ ID NO: 12 - protein, 134 aa, Mus musculus
EAKLQESGPVLVKPGASVKMSCKASGYTFTDYYMNWVKQSHGKSLEWIGVINPYNGDTSYNQKFKGKATLTVDKSSSTAYMELNSLTSEDSAVYYCARYYGSWFAYWGQGTLITVSTAKTTPPSVYPLAPRSSR

SEQ ID NO: 13 - protein, 356 aa, Mus musculus
EAKLQESGPVLVKPGASVKMSCKASGYTFTDYYMNWVKQSHGKSLEWIGVINPYNGDTSYNQKFKGKATLTVDKSSSTAYMELNSLTSEDSAVYYCARYYGSWFAYWGQGTLITVSTAKTTPPSVYPLAPRSSRGCKPCICTVPEVSSVFIFPPKPKDVLTITLTPKVTCVVVDISKDDPEVQFSWFVDDVEVHTAQTQPREEQFNSTFRSVSELPIMHQDWLNGKEFKCRVNSAAFPAPIEKTISKTKGRPKAPQVYTIPPPKEQMAKDKVSLTCMITDFFPEDITVEWQWNGQPAENYKNTQPIMDTDGSYFVYSKLNVQKSNWEAGNTFTCSVLHEGLHNHHTEKSLSHSPGK

SEQ ID NO: 14 - protein, 519 aa, Mus musculus
METDTLLLWVLLLWVPGSTGDIRRADIVMTQTTLSLPVSLGDQASISCRSSQSIVHSNGNTYLEWYLQKPGQSPKLLIYKVSNRFSGVPDRFSGSGSGTDFTLKISRVEAEDLGVYYCFQGSHVPYTFGGGTKLEIKRADAAPTVSGSGGGGSGGGGSGGGGSEAKLQESGPVLVKPGASVKMSCKASGYTFTDYYMNWVKQSHGKSLEWIGVINPYNGDTSYNQKFKGKATLTVDKSSSTAYMELNSLTSEDSAVYYCARYYGSWFAYWGQGTLITVSTAKTTPPSVYPLAPRSSRGCKPCICTVPEVSSVFIFPPKPKDVLTITLTPKVTCVVVDISKDDPEVQFSWFVDDVEVHTAQTQPREEQFNSTFRSVSELPIMHQDWLNGKEFKCRVNSAAFPAPIEKTISKTKGRPKAPQVYTIPPPKEQMAKDKVSLTCMITDFFPEDITVEWQWNGQPAENYKNTQPIMDTDGSYFVYSKLNVQKSNWEAGNTFTCSVLHEGLHNHHTEKSLSHSPGK

SEQ ID NO: 15 - DNA, 1560 bp, Mus musculus
atggaaactgatactctgctgctctgggtgctgctcctctgggtgcctggttcaactggggacattcgacgggctgacattgtgatgacccagaccacactgagcctgcccgtgtccctgggcgaccaggccagcatctcctgccggagctcccagtctatcgtgcacagcaacggaaacacatacctggagtggtatctgcagaagcctggccagtccccaaagctgctgatctacaaggtgtccaacaggttcagcggcgtgcctgaccgcttttctggaagcggctccggaacagatttcaccctgaagatcagcagggtggaggctgaggacctgggcgtgtactactgcttccagggatcccacgtgccttacacctttggcggaggcacaaagctggagatcaagagagccgatgctgctccaaccgtgtctggaagcggaggcgggggttctggaggcggtgggagcggtggcggagggtctgaggctaagctgcaggagagcggccccgtgctggtgaagcctggagccagcgtgaagatgtcctgtaaggcttctggatacaccttcacagactactacatgaactgggtgaagcagagccacggcaagtccctggagtggatcggagtgatcaacccttacaacggcgacacctcttacaaccagaagtttaagggcaaggccaccctgacagtggataagtctagctccaccgcttacatggagctgaacagcctgacatccgaggattctgccgtgtactactgtgctaggtactacggaagctggttcgcctactggggccagggaacactgatcaccgtgtccacagccaagaccacaccccctagcgtgtaccccctggctcctaggtctagcagaggctgcaagccatgcatctgtaccgtgcccgaggtgagcagcgtgttcatctttccacccaagcccaaggacgtgctgaccatcacactgacccctaaggtgacatgcgtggtggtggatatcagcaaggacgatccagaggtgcagttctcctggtttgtggacgatgtggaggtgcacaccgcccagacacagccaagggaggagcagttcaactccacctttagatccgtgtctgagctgcccatcatgcaccaggactggctgaacggaaaggagttcaagtgccgggtgaactccgccgcttttcctgctccaatcgagaagaccatctctaagacaaagggccgcccaaaggctccacaggtgtacaccatccctccacccaaggagcagatggctaaggataaggtgagcctgacctgtatgatcacagacttctttcccgaggatatcacagtggagtggcagtggaacggacagcctgccgagaactacaagaacacccagccaatcatggacacagatggctcttacttcgtgtacagcaagctgaacgtgcagaagtctaactgggaggctggcaacaccttcacctgcagcgtgctgcacgaaggtctccataatcaccacaccgaaaagagcctcagtcacagccctgggaaatga

SEQ ID NO: 16 - DNA, 1574 bp, Mus musculus
cttaagatggaaactgatactctgctgctctgggtgctgctcctctgggtgcctggttcaactggggacattcgacgggctgacattgtgatgacccagaccacactgagcctgcccgtgtccctgggcgaccaggccagcatctcctgccggagctcccagtctatcgtgcacagcaacggaaacacatacctggagtggtatctgcagaagcctggccagtccccaaagctgctgatctacaaggtgtccaacaggttcagcggcgtgcctgaccgcttttctggaagcggctccggaacagatttcaccctgaagatcagcagggtggaggctgaggacctgggcgtgtactactgcttccagggatcccacgtgccttacacctttggcggaggcacaaagctggagatcaagagagccgatgctgctccaaccgtgtctggaagcggaggcgggggttctggaggcggtgggagcggtggcggagggtctgaggctaagctgcaggagagcggccccgtgctggtgaagcctggagccagcgtgaagatgtcctgtaaggcttctggatacaccttcacagactactacatgaactgggtgaagcagagccacggcaagtccctggagtggatcggagtgatcaacccttacaacggcgacacctcttacaaccagaagtttaagggcaaggccaccctgacagtggataagtctagctccaccgcttacatggagctgaacagcctgacatccgaggattctgccgtgtactactgtgctaggtactacggaagctggttcgcctactggggccagggaacactgatcaccgtgtccacagccaagaccacaccccctagcgtgtaccccctggctcctaggtctagcagaggctgcaagccatgcatctgtaccgtgcccgaggtgagcagcgtgttcatctttccacccaagcccaaggacgtgctgaccatcacactgacccctaaggtgacatgcgtggtggtggatatcagcaaggacgatccagaggtgcagttctcctggtttgtggacgatgtggaggtgcacaccgcccagacacagccaagggaggagcagttcaactccacctttagatccgtgtctgagctgcccatcatgcaccaggactggctgaacggaaaggagttcaagtgccgggtgaactccgccgcttttcctgctccaatcgagaagaccatctctaagacaaagggccgcccaaaggctccacaggtgtacaccatccctccacccaaggagcagatggctaaggataaggtgagcctgacctgtatgatcacagacttctttcccgaggatatcacagtggagtggcagtggaacggacagcctgccgagaactacaagaacacccagccaatcatggacacagatggctcttacttcgtgtacagcaagctgaacgtgcagaagtctaactgggaggctggcaacaccttcacctgcagcgtgctgcacgaaggtctccataatcaccacaccgaaaagagcctcagtcacagccctgggaaatgaggcgcgcc

SEQ ID NO: 17 - DNA, 1484 bp, Homo sapiens
cttaagatggaaactgacaccctgctgctgtgggtcctgctgctgtgggtgcctggatccaccggcgatatcgtgctgacccagtctcctggcacactgagtctgtcaccaggggagcgagcaacactgtcttgtagagccagccagtctgtgggaagctcctacctggcttggtatcagcagaagccaggccaggcacccaggctgctgatctacggagccttcagccgggccactggcattccagacaggttctctggaagtggctcagggaccgacttcaccctgaccatcagccgactggagcccgaagacttcgccgtgtactattgccagcagtacggctctagtccttggacttttggacagggcaccaaagtggagatcaagcgcggcgggggaggctctgggggaggcgggagtggaggcgggggatcacaggtccagctggtggaaagcggcgggggagtggtccagccaggccggagcctgcggctgagctgcgccgcttcaggattcacattttcaagctataccatgcactgggtccggcaggcaccagggaagggactggagtgggtgaccttcatcagctatgacggcaacaacaagtattacgctgattccgtgaaagggaggtttaccattagccgcgacaactccaaaaatacactgtacctgcagatgaacagcctgcgggccgaggatactgctatctactattgcgcaagaaccgggtggctgggacccttcgactattggggccaggggactctggtcaccgtgtcctctgataagacacacacatgccctccctgtcctgcaccagagctgctgggcgggccatccgtgttcctgtttccacccaagcctaaagacaccctgatgatcagccggacacctgaagtcacttgcgtggtcgtggacgtgagtcacgaggatccagaagtcaagtttaactggtacgtggatggcgtcgaggtgcataatgccaagaccaaacctcgcgaggaacagtacaatagcacatatcgagtcgtgtccgtcctgactgtgctgcatcaggattggctgaacggcaaagagtataagtgcaaagtgagcaataaggcactgcctgccccaatcgagaaaacaatttccaaggctaaaggccagcccagggaacctcaggtgtacactctgcctccaagtcgcgaggaaatgaccaagaaccaggtgagcctgacctgtctggtgaaagggttctatccatcagacattgcagtggagtgggaaagcaatggacagcccgaaaacaattacaagaccacaccccctgtgctggacagcgatggctccttctttctgtattctaagctgactgtggataaaagtcgctggcagcaggggaacgtctttagctgttccgtgatgcatgaggctctgcacaatcattacacacagaagtctctgagtctgtcacccggcaaatgaggcgcgcc

SEQ ID NO: 18 - DNA, 426 bp, Mus musculus
atgtggctgcagaatttacttttcctgggcattgtggtctacagcctctcagcacccacccgctcacccatcactgtcacccggccttggaagcatgtagaggccatcaaagaagccctgaacctcctggatgacatgcctgtcacattgaatgaagaggtagaagtcgtctctaacgagttctccttcaagaagctaacatgtgtgcagacccgcctgaagatattcgagcagggtctacggggcaatttcaccaaactcaagggcgccttgaacatgacagccagctactaccagacatactgccccccaactccggaaacggactgtgaaacacaagttaccacctatgcggatttcatagacagccttaaaacctttctgactgatatcccctttgaatgcaaaaaaccagtccaaaaatga

SEQ ID NO: 19 - DNA, 426 bp, Mus musculus
atgtggctccagaacctcctcttcctcggtatcgtcgtgtattcactctccgcacctactcgctcacctatcactgtcaccagaccctggaagcacgtggaggccatcaaggaggctctgaacctgctggacgatatgccagtgaccctgaacgaggaggtggaggtggtgagcaacgagttctcctttaagaagctgacctgcgtgcagacaaggctgaagatcttcgagcagggcctgagaggaaactttaccaagctgaagggcgccctgaacatgaccgcttcttactaccagacatactgcccccctacccccgagacagactgtgagacacaggtgaccacatacgccgacttcattgatagcctgaaaacattcctgaccgacattccatttgagtgtaagaagcccgtccagaagtaa

SEQ ID NO: 20 - DNA, 435 bp, Homo sapiens
atgtggctgcagagcctgctgctcttgggcactgtggcctgcagcatctctgcacccgcccgctcgcccagccccagcacgcagccctgggagcatgtgaatgccatccaggaggcccggcgtctcctgaacctgagtagagacactgctgctgagatgaatgaaacagtagaagtcatctcagaaatgtttgacctccaggagccgacctgcctacagacccgcctggagctgtacaagcagggcctgcggggcagcctcaccaagctcaagggccccttgaccatgatggccagccactacaagcagcactgccctccaaccccggaaacttcctgtgcaacccagattatcacctttgaaagtttcaaagagaacctgaaggactttctgcttgtcatcccctttgactgctgggagccagtccaggagtga

SEQ ID NO: 21 - DNA, 435 bp, Homo sapiens
atgtggctgcagtccctgctgctgctgggcaccgtcgcctgttctatttccgcacccgcaaggtcaccaagtccatctactcagccttgggagcacgtgaacgcaatccaggaggcacggcggctgctgaacctgagccgggacaccgccgccgagatgaacgagacagtggaagtgatcagcgagatgttcgatctgcaggagcccacctgcctgcagacaaggctggagctgtacaagcagggcctgcgcggctctctgaccaagctgaagggcccactgacaatgatggccagccactataagcagcactgcccccctacccccgagacaagctgtgccacccagatcatcacattcgagtcctttaaggagaacctgaaggattttctgctggtcattccatttgattgttgggagcccgtccaggagtaa

SEQ ID NO: 22 - protein, 141 aa, Mus musculus
MWLQNLLFLGIVVYSLSAPTRSPITVTRPWKHVEAIKEALNLLDDMPVTLNEEVEVVSNEFSFKKLTCVQTRLKIFEQGLRGNFTKLKGALNMTASYYQTYCPPTPETDCETQVTTYADFIDSLKTFLTDIPFECKKPVQK

SEQ ID NO: 23 - protein, 144 aa, Homo sapiens
MWLQSLLLLGTVACSISAPARSPSPSTQPWEHVNAIQEARRLLNLSRDTAAEMNETVEVISEMFDLQEPTCLQTRLELYKQGLRGSLTKLKGPLTMMASHYKQHCPPTPETSCATQIITFESFKENLKDFLLVIPFDCWEPVQE

SEQ ID NO: 24 - DNA, 2010 bp, Gibbon leukemia virus
atggtattgctgcctgggtccatgcttctcacctcaaacctgcaccaccttcggcaccagatgagtcctgggagctggaaaagactgatcatcctcttaagctgcgtattcggcggcggcgggacgagtctgcaaaataagaacccccaccagcccatgaccctcacttggcaggtactgtcccaaactggagacgttgtctgggatacaaaggcagtccagcccccttggacttggtggcccacacttaaacctgatgtatgtgccttggcggctagtcttgagtcctgggatatcccgggaaccgatgtctcgtcctctaaacgagtcagacctccggactcagactatactgccgcttataagcaaatcacctggggagccatagggtgcagctaccctcgggctaggactagaatggcaagctctaccttctacgtatgtccccgggatggccggaccctttcagaagctagaaggtgcggggggctagaatccctatactgtaaagaatgggattgtgagaccacggggaccggttattggctatctaaatcctcaaaagacctcataactgtaaaatgggaccaaaatagcgaatggactcaaaaatttcaacagtgtcaccagaccggctggtgtaacccccttaaaatagatttcacagacaaaggaaaattatccaaggactggataacgggaaaaacctggggattaagattctatgtgtctggacatccaggcgtacagttcaccattcgcttaaaaatcaccaacatgccagctgtggcagtaggtcctgacctcgtccttgtggaacaaggacctcctagaacgtccctcgctctcccacctcctcttcccccaagggaagcgccaccgccatctctccccgactctaactccacagccctggcgactagtgcacaaactcccacggtgagaaaaacaattgttaccctaaacactccgcctcccaccacaggcgacagactttttgatcttgtgcagggggccttcctaaccttaaatgctaccaacccaggggccactgagtcttgctggctttgtttggccatgggccccccttattatgaagcaatagcctcatcaggagaggtcgcctactccaccgaccttgaccggtgccgctgggggacccaaggaaagctcaccctcactgaggtctcaggacacgggttgtgcataggaaaggtgccctttacccatcagcatctctgcaatcagaccctatccatcaattcctccggagaccatcagtatctgctcccctccaaccatagctggtgggcttgcagcactggcctcaccccttgcctctccacctcagtttttaatcagactagagatttctgtatccaggtccagctgattcctcgcatctattactatcctgaagaagttttgttacaggcctatgacaattctcaccccaggactaaaagagaggctgtctcacttaccctagctgttttactggggttgggaatcacggcgggaataggtactggttcaactgccttaattaaaggacctatagacctccagcaaggcctgacaagcctccagatcgccatagatgctgacctccgggccctccaagactcagtcagcaagttagaggactcactgacttccctgtccgaggtagtgctccaaaataggagaggccttgacttgctgtttctaaaagaaggtggcctctgtgcggccctaaaggaagagtgctgtttttacatagaccactcaggtgcagtacgggactccatgaaaaaactcaaagaaaaactggataaaagacagttagagcgccagaaaagccaaaactggtatgaaggatggttcaataactccccttggttcactaccctgctatcaaccatcgctgggcccctattactcctccttctgttgctcatcctcgggccatgcatcatcaataagttagttcaattcatcaatgataggataagtgcagttaaaatttaa

SEQ ID NO: 25 - DNA, 2013 bp, Gibbon leukemia virus
accatggtcctgctgcctgggtctatgctgctgacttctaacctgcaccacctgcgacaccagatgtctcccggctcatggaaacggctgatcatcctgctgagctgcgtgttcggaggaggaggcacctccctgcagaacaagaatcctcaccagccaatgaccctgacatggcaggtgctgtcccagacaggcgacgtggtgtgggataccaaggcagtgcagccaccttggacatggtggcccaccctgaagcctgacgtgtgcgccctggccgcctccctggagtcttgggacatccccggcacagacgtgagcagcagcaagagggtgagaccacccgactctgattatacagccgcctacaagcagatcacctggggcgccatcggctgtagctatcctcgggcccgcacaaggatggccagctccaccttttacgtgtgcccacgcgacggaaggaccctgtctgaggcaaggagatgtggcggcctggagagcctgtattgcaaggagtgggattgtgagaccacaggcacaggctactggctgtctaagtctagcaaggacctgatcaccgtgaagtgggatcagaacagcgagtggacacagaagttccagcagtgccaccagaccggctggtgtaatcccctgaagatcgactttacagataagggcaagctgtccaaggactggatcaccggcaagacatggggcctgagattctacgtgtctggccaccctggcgtgcagtttacaatccggctgaagatcaccaacatgccagcagtggcagtgggaccagacctggtgctggtggagcagggacctccacgcacctccctggccctgccccctccactgccccctagggaggccccaccccctagcctgcccgattctaacagcacagccctggccacctccgcccagacccctacagtgcgcaagaccatcgtgacactgaataccccaccccctaccacaggcgacaggctgttcgatctggtgcagggcgcctttctgacactgaacgccaccaatcctggcgcaaccgagagctgctggctgtgcctggctatgggcccaccctactatgaggcaatcgcctcctctggagaggtggcatattccacagacctggatagatgcagatggggcacccagggcaagctgaccctgacagaggtgtctggccacggcctgtgcatcggcaaggtgccattcacacaccagcacctgtgcaaccagaccctgagcatcaatagctccggcgaccaccagtacctgctgccaagcaaccactcctggtgggcatgctccacaggactgaccccatgtctgagcaccagcgtgttcaaccagaccagagacttttgtatccaggtgcagctgatccctcggatctactattacccagaggaggtgctgctgcaggcctatgataattcccacccaagaacaaagagggaggccgtgtctctgaccctggccgtgctgctgggactgggaatcacagcaggaatcggcacaggcagcaccgccctgatcaagggaccaatcgacctgcagcagggactgacctccctgcagatcgccatcgacgccgatctgagagccctgcaggacagcgtgtccaagctggaggattctctgacctctctgagcgaggtggtgctgcagaacaggaggggcctggacctgctgttcctgaaggagggaggactgtgcgccgccctgaaggaggagtgctgtttttatatcgaccactctggcgccgtgcgggatagcatgaagaagctgaaggagaagctggataagcgccagctggagaggcagaagagccagaattggtacgagggctggttcaacaattccccctggtttaccacactgctgtctaccatcgcaggacctctgttattactgctgctgctgctgatcctgggcccatgtatcatcaacaagctggtgcagtttatcaacgaccgaatctccgcagtgaaaatctaa

SEQ ID NO: 26 - protein, 669 aa, Gibbon leukemia virus
MVLLPGSMLLTSNLHHLRHQMSPGSWKRLIILLSCVFGGGGTSLQNKNPHQPMTLTWQVLSQTGDVVWDTKAVQPPWTWWPTLKPDVCALAASLESWDIPGTDVSSSKRVRPPDSDYTAAYKQITWGAIGCSYPRARTRMASSTFYVCPRDGRTLSEARRCGGLESLYCKEWDCETTGTGYWLSKSSKDLITVKWDQNSEWTQKFQQCHQTGWCNPLKIDFTDKGKLSKDWITGKTWGLRFYVSGHPGVQFTIRLKITNMPAVAVGPDLVLVEQGPPRTSLALPPPLPPREAPPPSLPDSNSTALATSAQTPTVRKTIVTLNTPPPTTGDRLFDLVQGAFLTLNATNPGATESCWLCLAMGPPYYEAIASSGEVAYSTDLDRCRWGTQGKLTLTEVSGHGLCIGKVPFTHQHLCNQTLSINSSGDHQYLLPSNHSWWACSTGLTPCLSTSVFNQTRDFCIQVQLIPRIYYYPEEVLLQAYDNSHPRTKREAVSLTLAVLLGLGITAGIGTGSTALIKGPIDLQQGLTSLQIAIDADLRALQDSVSKLEDSLTSLSEVVLQNRRGLDLLFLKEGGLCAALKEECCFYIDHSGAVRDSMKKLKEKLDKRQLERQKSQNWYEGWFNNSPWFTTLLSTIAGPLLLLLLLLILGPCIINKLVQFINDRISAVKI

SEQ ID NO: 27 - DNA, 759 bp, Artificial Sequence
  Human-Mouse hybrid
atgatcgagacctacaatcagacaagcccacggtccgccgcaaccggactgcctatcagcatgaagatcttcatgtacctgctgaccgtgtttctgatcacacagatgatcggctccgccctgttcgccgtgtatctgcacaggagactggacaagatcgaggatgagcgcaatctgcacgaggacttcgtgtttatgaagaccatccagcggtgcaacacaggcgagaggagcctgtctctgctgaattgtgaggagatcaagtcccagttcgagggctttgtgaaggatatcatgctgaacaaggaggagacaaagaaggacgaggatccacagatcgcagcacacgtggtgtccgaggcaaactctaatgccgccagcgtgctgcagtgggccaagaagggctactataccatgaagtctaacctggtgacactggagaatggcaagcagctgaccgtgaagaggcagggcctgtactatatctatgcccaggtgacattctgctctaacagagaggcaagctcccaggcacccttcatcgtgggactgtggctgaagccctctagcggcagcgagaggatcctgctgaaggccgccaatacccactcctctagccagctgtgcgagcagcagtccatccacctgggaggcgtgttcgagctgcagcctggagccagcgtgttcgtgaacgtgacagacccatctcaggtgagccacggcaccggcttcacaagctttggcctgctgaagctgtga

SEQ ID NO: 28 - protein, 252 aa, Artificial Sequence
  Human-Mouse hybrid
MIETYNQTSPRSAATGLPISMKIFMYLLTVFLITQMIGSALFAVYLHRRLDKIEDERNLHEDFVFMKTIQRCNTGERSLSLLNCEEIKSQFEGFVKDIMLNKEETKKDEDPQIAAHVVSEANSNAASVLQWAKKGYYTMKSNLVTLENGKQLTVKRQGLYYIYAQVTFCSNREASSQAPFIVGLWLKPSSGSERILLKAANTHSSSQLCEQQSIHLGGVFELQPGASVFVNVTDPSQVSHGTGFTSFGLLKL

SEQ ID NO: 29 - DNA, 1416 bp, Homo sapiens
atgctgccctttctgagcatgctggtgctgctggtgcagcctctgggaaacctgggagccgagatgaagagcctgtcccagagatctgtgcctaacacctgcacactggtcatgtgcagccccaccgagaatggactgcctggaagggacggaagggatggaagggagggccctcggggcgagaagggcgacccaggactgcctggaccaatgggactgagcggactgcagggaccaacaggacctgtgggaccaaagggagagaacggatccgccggagagccaggccctaagggcgagaggggcctgtctggcccccctggcctgccaggcatcccaggccccgccggcaaggagggcccatccggcaagcagggcaatatcggcccccagggcaagcctggcccaaagggcgaggcaggaccaaagggagaagtgggagcacctggcatgcagggatccaccggagcaaagggatctacaggaccaaagggcgagcgcggcgccccaggcgtgcagggcgcccccggcaatgcaggagcagcaggaccagcaggacctgcaggcccacagggcgcccctggctctaggggcccacccggcctgaagggcgacaggggagtgcctggcgataggggcatcaagggagagagcggactgccagattccgccgccctgaggcagcagatggaggccctgaagggcaagctgcagaggctggaggtggccttctcccactaccagaaggccgccctgtttccagacggccacaggagactggacaagatcgaggatgagcgcaacctgcacgaggatttcgtgtttatgaagaccatccagagatgcaacacaggcgagcggtctctgagcctgctgaattgtgaggagatcaagtctcagttcgagggctttgtgaaggacatcatgctgaacaaggaggagaccaagaaggagaatagcttcgagatgcagaagggcgatcagaatccccagatcgcagcacacgtgatcagcgaggcaagctccaagaccacatccgtgctgcagtgggccgagaagggctactataccatgtccaacaatctggtgacactggagaacggcaagcagctgaccgtgaagagacagggcctgtactatatctatgcccaggtgacattctgctctaatcgggaggcctctagccaggccccttttatcgcctctctgtgcctgaagagcccaggcagattcgagcggatcctgctgagggccgccaacacccactcctctgccaagccatgcggacagcagagcatccacctgggaggcgtgttcgagctgcagccaggagcctccgtgtttgtgaatgtgacagacccatcccaggtgtctcacggaaccggcttcacatcctttggcctgctgaagctgtga

SEQ ID NO: 30 - protein, 471 aa, Homo sapiens
MLPFLSMLVLLVQPLGNLGAEMKSLSQRSVPNTCTLVMCSPTENGLPGRDGRDGREGPRGEKGDPGLPGPMGLSGLQGPTGPVGPKGENGSAGEPGPKGERGLSGPPGLPGIPGPAGKEGPSGKQGNIGPQGKPGPKGEAGPKGEVGAPGMQGSTGAKGSTGPKGERGAPGVQGAPGNAGAAGPAGPAGPQGAPGSRGPPGLKGDRGVPGDRGIKGESGLPDSAALRQQMEALKGKLQRLEVAFSHYQKAALFPDGHRRLDKIEDERNLHEDFVFMKTIQRCNTGERSLSLLNCEEIKSQFEGFVKDIMLNKEETKKENSFEMQKGDQNPQIAAHVISEASSKTTSVLQWAEKGYYTMSNNLVTLENGKQLTVKRQGLYYIYAQVTFCSNREASSQAPFIASLCLKSPGRFERILLRAANTHSSAKPCGQQSIHLGGVFELQPGASVFVNVTDPSQVSHGTGFTSFGLLKL

SEQ ID NO: 31 - DNA, 1412 bp, Mus musculus
atgctgcccttcctgagcatgctggtgctgctggtgcagcctctgggcaatctgggcgccgagatgaagtccctgtctcagaggagcgtgccaaacacctgcacactggtcatgtgctctccaaccgagaatggactgccaggaagggacggaagagatggaagggagggaccaaggggagagaagggcgaccctggactgcctggaccaatgggactgtccggactgcagggaccaacaggccctgtgggaccaaagggagagaatggaagcgccggagagccaggacctaagggagagaggggcctgtccggcccccctggcctgcctggcatcccaggccccgccggcaaggagggcccttctggcaagcagggcaacatcggaccacagggcaagcctggaccaaagggagaggcaggaccaaagggagaagtgggagcacccggcatgcagggcagcaccggagcaaagggatccaccggccctaagggagagagaggagcacctggagtgcagggcgccccaggcaatgcaggagcagcaggaccagcaggacctgcaggcccacagggcgccccaggcagccggggcccacccggcctgaagggcgacaggggagtgccaggcgataggggcatcaagggagagtccggactgccagactctgccgccctgaggcagcagatggaggccctgaagggcaagctgcagaggctggaggtggccttctcccactaccagaaggccgccctgtttccagacggacacaggagactggataaggtggaggaggaggtgaacctgcacgaggatttcgtgttcatcaagaagctgaagaggtgcaacaagggcgagggcagcctgtccctgctgaattgtgaggagatgcggcgccagttcgaggacctggtgaaggatatcaccctgaacaaggaggagaagaaggagaattcttttgagatgcagaggggcgacgaggatcctcagatcgcagcacacgtggtgtccgaggcaaactctaatgccgccagcgtgctgcagtgggccaagaagggctactataccatgaagtctaacctggtcatgctggagaatggcaagcagctgacagtgaagagagagggcctgtactacgtgtacacccaggtgacattctgcagcaacagagagcccagctcccagcggccttttatcgtgggcctgtggctgaagccctctatcggaagcgagaggatcctgctgaaggcagccaatacccactctagctcccagctgtgcgagcagcagtccgtgcacctgggaggcgtgttcgagctgcaggcaggagcaagcgtgttcgtgaacggacagaggccagccaggtcatccacagagtgggcttctctagctttggcctgctgaagctgtga

SEQ ID NO: 32 - protein, 470 aa, Mus musculus
MLPFLSMLVLLVQPLGNLGAEMKSLSQRSVPNTCTLVMCSPTENGLPGRDGRDGREGPRGEKGDPGLPGPMGLSGLQGPTGPVGPKGENGSAGEPGPKGERGLSGPPGLPGIPGPAGKEGPSGKQGNIGPQGKPGPKGEAGPKGEVGAPGMQGSTGAKGSTGPKGERGAPGVQGAPGNAGAAGPAGPAGPQGAPGSRGPPGLKGDRGVPGDRGIKGESGLPDSAALRQQMEALKGKLQRLEVAFSHYQKAALFPDGHRRLDKVEEEVNLHEDFVFIKKLKRCNKGEGSLSLLNCEEMRRQFEDLVKDITLNKEEKKENSFEMQRGDEDPQIAAHVVSEANSNAASVLQWAKKGYYTMKSNLVMLENGKQLTVKREGLYYVYTQVTFCSNREPSSQRPFIVGLWLKPSIGSERILLKAANTHSSSQLCEQQSVHLGGVFELQAGASVFVNVTEASQVIHRVGFSSFGLLKL

SEQ ID NO: 33 - DNA, 786 bp, Homo sapiens
atgatcgaaacatacaaccaaacttctccccgatctgcggccactggactgcccatcagcatgaaaatttttatgtatttacttactgtttttcttatcacccagatgattgggtcagcactttttgctgtgtatcttcatagaaggttggacaagatagaagatgaaaggaatcttcatgaagattttgtattcatgaaaacgatacagagatgcaacacaggagaaagatccttatccttactgaactgtgaggagattaaaagccagtttgaaggctttgtgaaggatataatgttaaacaaagaggagacgaagaaagaaaacagctttgaaatgcaaaaaggtgatcagaatcctcaaattgcggcacatgtcataagtgaggccagcagtaaaacaacatctgtgttacagtgggctgaaaaaggatactacaccatgagcaacaacttggtaaccctggaaaatgggaaacagctgaccgttaaaagacaaggactctattatatctatgcccaagtcaccttctgttccaatcgggaagcttcgagtcaagctccatttatagccagcctctgcctaaagtcccccggtagattcgagagaatcttactcagagctgcaaatacccacagttccgccaaaccttgcgggcaacaatccattcacttgggaggagtatttgaattgcaaccaggtgcttcggtgtttgtcaatgtgactgatccaagccaagtgagccatggcactggcttcacgtcctttggcttactcaaactctga

SEQ ID NO: 34 - protein, 261 aa, Homo sapiens
MIETYNQTSPRSAATGLPISMKIFMYLLTVFLITQMIGSALFAVYLHRRLDKIEDERNLHEDFVFMKTIQRCNTGERSLSLLNCEEIKSQFEGFVKDIMLNKEETKKENSFEMQKGDQNPQIAAHVISEASSKTTSVLQWAEKGYYTMSNNLVTLENGKQLTVKRQGLYYIYAQVTFCSNREASSQAPFIASLCLKSPGRFERILLRAANTHSSAKPCGQQSIHLGGVFELQPGASVFVNVTDPSQVSHGTGFTSFGLLKL

SEQ ID NO: 35 - DNA, 783 bp, Mus musculus
atgatagaaacatacagccaaccttcccccagatccgtggcaactggacttccagcgagcatgaagatttttatgtatttacttactgttttccttatcacccaaatgattggatctgtgctttttgctgtgtatcttcatagaagattggataaggtcgaagaggaagtaaaccttcatgaagattttgtattcataaaaaagctaaagagatgcaacaaaggagaaggatctttatccttgctgaactgtgaggagatgagaaggcaatttgaagaccttgtcaaggatataacgttaaacaaagaagagaaaaaagaaaacagctttgaaatgcaaagaggtgatgaggatcctcaaattgcagcacacgttgtaagcgaagccaacagtaatgcagcatccgttctacagtgggccaagaaaggatattataccatgaaaagcaacttggtaatgcttgaaaatgggaaacagctgacggttaaaagagaaggactctattatgtctacactcaagtcaccttctgctctaatcgggagccttcgagtcaacgcccattcatcgtcggcctctggctgaagcccagcagtggatctgagagaatcttactcaaggcggcaaatacccacagttcctcccagctttgcgagcagcagtctgttcacttgggcggagtgtttgaattacaagctggtgcttctgtgtttgtcaacgtgactgaagcaagccaagtgatccacagagttggcttctcatcttttggcttactcaaactctga

SEQ ID NO: 36 - protein, 260 aa, Mus musculus
MIETYSQPSPRSVATGLPASMKIFMYLLTVFLITQMIGSVLFAVYLHRRLDKVEEEVNLHEDFVFIKKLKRCNKGEGSLSLLNCEEMRRQFEDLVKDITLNKEEKKENSFEMQRGDEDPQIAAHVVSEANSNAASVLQWAKKGYYTMKSNLVMLENGKQLTVKREGLYYVYTQVTFCSNREPSSQRPFIVGLWLKPSSGSERILLKAANTHSSSQLCEQQSVHLGGVFELQAGASVFVNVTEASQVIHRVGFSSFGLLKL

SEQ ID NO: 37 - DNA, 632 bp, Artificial Sequence
  CMV promoter
gttgacattgattattgactagttattaatagtaatcaattacggggtcattagttcatagcccatatatggagttccgcgttacataacttacggtaaatggcccgcctggctgaccgcccaacgacccccgcccattgacgtcaataatgacgtatgttcccatagtaacgccaatagggactttccattgacgtcaatgggtggagtatttacggtaaactgcccacttggcagtacatcaagtgtatcatatgccaagtacgccccctattgacgtcaatgacggtaaatggcccgcctggcattatgcccagtacatgaccttatgggactttcctacttggcagtacatctacgtattagtcatcgctattaccatggtgatgcggttttggcagtacatcaatgggcgtggatagcggtttgactcacggggatttccaagtctccaccccattgacgtcaatgggagtttgttttggcaccaaaatcaacgggactttccaaaatgtcgtaacaactccgccccattgacgcaaatgggcggtaggcgtgtacggtgggaggtctatataagcagagctctctggctaactagagaacccactgcttactggcttatcgaaatt

SEQ ID NO: 38 - DNA, 394 bp, Artificial Sequence
  RSV promoter
tgtacgggccagatatacgcgtatctgaggggactagggtgtgtttaggcgaaaagcggggcttcggttgtacgcggttaggagtcccctcaggatatagtagtttcgcttttgcatagggagggggaaatgtagtcttatgcaatacacttgtagtcttgcaacatggtaacgatgagttagcaacatgccttacaaggagagaaaaagcaccgtgcatgccgattggtggaagtaaggtggtacgatcgtgccttattaggaaggcaacagacaggtctgacatggattggacgaaccactgaattccgcattgcagagataattgtatttaagtgcctagctcgatacaataaacgccatttgaccattcaccacattggtgtgcacctcc

SEQ ID NO: 39 - DNA, 188 bp, Artificial Sequence
  BGH polyA
ctgtgccttctagttgccagccatctgttgtttgcccctcccccgtgccttccttgaccctggaaggtgccactcccactgtcctttcctaataaaatgaggaaattgcatcgcattgtctgagtaggtgtcattctattctggggggtggggtggggcaggacagcaagggggaggattgggaagac

SEQ ID NO: 40 - DNA, 249 bp, Artificial Sequence
  SV40 late polyA
gacatgataagatacattgatgagtttggacaaaccacaactagaatgcagtgaaaaaaatgctttatttgtgaaatttgtgatgctattgctttatttgtgaaatttgtgatgctattgctttatttgtaaccattataagctgcaataaacaagttaacaacaacaattgcattcattttatgtttcaggttcagggggaggtgtgggaggttttttaaagcaagtaaaacctctacaaatgtggta

SEQ ID NO: 41 - DNA, 99 bp, Artificial Sequence
  Rabbit beta-globulin polyA
gacctctggctaataaaggaaatttattttcattgcaatagtgtgttggaattttttgtgtctctcactcggaaggacatatgggagggcaaatcattt

SEQ ID NO: 42 - DNA, 723 bp, Artificial Sequence
  GFP
accatggtgagcaagggcgaggagctgttcaccggggtggtgcccatcctggtcgagctggacggcgacgtaaacggccacaagttcagcgtgtccggcgagggcgagggcgatgccacctacggcaagctgaccctgaagttcatctgcaccaccggcaagctgcccgtgccctggcccaccctcgtgaccaccctgacctacggcgtgcagtgcttcagccgctaccccgaccacatgaagcagcacgacttcttcaagtccgccatgcccgaaggctacgtccaggagcgcaccatcttcttcaaggacgacggcaactacaagacccgcgccgaggtgaagttcgagggcgacaccctggtgaaccgcatcgagctgaagggcatcgacttcaaggaggacggcaacatcctggggcacaagctggagtacaactacaacagccacaacgtctatatcatggccgacaagcagaagaacggcatcaaggtgaacttcaagatccgccacaacatcgaggacggcagcgtgcagctcgccgaccactaccagcagaacacccccatcggcgacggccccgtgctgctgcccgacaaccactacctgagcacccagtccgccctgagcaaagaccccaacgagaagcgcgatcacatggtcctgctggagttcgtgaccgccgccgggatcactctcggcatggacgagctgtacaagtaa

SEQ ID NO: 43 - DNA, 454 bp, Artificial Sequence
  MoMuLV LTR
ttaattaagtaacgccattttgcaaggcatggaaaaatacataactgagaatagagaagttcagatcaaggtcaggaacagatggaacagctgaatatgggccaaacaggatatctgtggtaagcagttcctgccccggctcagggccaagaacagatggaacagctgaatatgggccaaacaggatatctgtggtaagcagttcctgccccggctcagggccaagaacagatggtccccagatgcggtccagccctcagcagtttctagagaaccatcagatgtttccagggtgccccaaggacctgaaatgaccctgtgccttatttgaactaaccaatcagttcgcttctcgcttctgttcgcgcgcttctgctccccgagctcaataaaagagcccacaacccctcactcggggcgccagtcctccgattgactgagtcgcccgcttaag

SEQ ID NO: 44 - DNA, 1349 bp, Artificial Sequence
  EF1alpha promoter
ttaattaagagtaattcatacaaaaggactcgcccctgccttggggaatcccagggaccgtcgttaaactcccactaacgtagaacccagagatcgctgcgttcccgccccctcacccgcccgctctcgtcatcactgaggtggagaagagcatgcgtgaggctccggtgcccgtcagtgggcagagcgcacatcgcccacagtccccgagaagttggggggaggggtcggcaattgaaccggtgcctagagaaggtggcgcggggtaaactgggaaagtgatgtcgtgtactggctccgcctttttcccgagggtgggggagaaccgtatataagtgcagtagtcgccgtgaacgttctttttcgcaacgggtttgccgccagaacacaggtaagtgccgtgtgtggttcccgcgggcctggcctctttacgggttatggcccttgcgtgccttgaattacttccacgcccctggctgcagtacgtgattcttgatcccgagcttcgggttggaagtgggtgggagagttcgaggccttgcggttaaggagccccttcgcctcgtgcttgagttgaggcctggcttgggcgctggggccgccgcgtgcgaatctggtggcaccttcgcgcctgtctcgctgctttcgataagtctctagccatttaaaatttttgatgacctgctgcgacgctttttttctggcaagatagtcttgtaaatgcgggccaagatctgcacactggtatttcggtttttggggccgcgggcggcgacggggcccgtgcgtcccagcgcacatgttcggcgaggcggggcctgcgagcgcggccaccgagaatcggacgggggtagtctcaagctggccggcctgctctggtgcctggcctcgcgccgccgtgtatcgccccgccctgggcggcaaggctggcccggtcggcaccagttgcgtgagcggaaagatggccgcttcccggccctgctgcagggagctcaaaatggaggacgcggcgctcgggagagcgggcgggtgagtcacccacacaaaggaaaagggcctttccgtcctcagccgtcgcttcatgtgactccacggagtaccgggcgccgtccaggcacctcgattagttctcgagcttttggagtacgtcgtctttaggttggggggaggggttttatgcgatggagtttccccacactgagtgggtggagactgaagttaggccagcttggcacttgatgtaattctccttggaatttgccctttttgagtttggatcttggttcattctcaagcctcagacagtggttcaaagtttttttcttccatttcaggtgtcgtgacttaag

SEQ ID NO: 45 - DNA, 345 bp, Artificial Sequence
  SV40 enhancer promoter
gctgtggaatgtgtgtcagttagggtgtggaaagtccccaggctccccagcaggcagaagtatgcaaagcatgcatctcaattagtcagcaaccaggtgtggaaagtccccaggctccccagcaggcagaagtatgcaaagcatgcatctcaattagtcagcaaccatagtcccgcccctaactccgcccatcccgcccctaactccgcccagttccgcccattctccgccccatggctgactaattttttttatttatgcagaggccgaggccgcctcggcctctgagctattccagaagtagtgaggaggcttttttggaggcctaggcttttgcaaaaagct

SEQ ID NO: 46 - DNA, 481 bp, Artificial Sequence
  HGH polyA
gacgggtggcatccctgtgacccctccccagtgcctctcctggccctggaagttgccactccagtgcccaccagccttgtcctaataaaattaagttgcatcattttgtctgactaggtgtccttctataatattatggggtggaggggggtggtatggagcaaggggcaagttgggaagacaacctgtagggcctgcggggtctattgggaaccaagctggagtgcagtggcacaatcttggctcactgcaatctccgcctcctgggttcaagcgattctcctgcctcagcctcccgagttgttgggattccaggcatgcatgaccaggctcagctaatttttgtttttttggtagagacggggtttcaccatattggccaggctggtctccaactcctaatctcaggtgatctacccaccttggcctcccaaattgctgggattacaggcgtgaaccactgctcccttccctgtccttt